European Patent Specification EP 3 673 085 B1, published March 11, 2026. Title: ENZYME SCREENING METHODS. Applicant: Roche Diagnostics Gmbh F. Hoffmann-La Roche Ag Roche Sequencing Solutions, Inc. President and Fellows of Harvard College. The sequence listing filed with the application follows.

SEQUENCE LISTING (3 sequences)

SEQ ID NO: 1 - DNA, 58 bp, Artificial Sequence
  Molecular barcode sequence
cagtcagtatttcccaaaccctttaaaagggtttgggaaaaaaaacggaggaggagga

SEQ ID NO: 2 - DNA, 58 bp, Artificial Sequence
  Molecular barcode sequence
cagtcagtaaaaccctttccctttaaaagggaaagggtttaaaaacggaggaggagga

SEQ ID NO: 3 - DNA, 58 bp, Artificial Sequence
  Molecular barcode sequence
cagtcagtatttccctttccctttaaaagggaaagggaaaaaaaacggaggaggagga